European Patent Application EP 4 397 776 A2, published July 10, 2024. Title: Method for classifying a patient's responsiveness to immune checkpoint inhibitor therapy. Applicant: Eberhard Karls Universität, Medizinische Fakultät. The sequence listing filed with the application follows.

SEQUENCE LISTING (10 sequences)

SEQ ID NO: 1 - DNA, 21 bp, synthetic construct
  misc_feature 1..21: note = None
  source 1..21: mol_type = other DNA
gcgtcgtggtggtcgcacagg

SEQ ID NO: 2 - DNA, 21 bp, synthetic construct
  misc_feature 1..21: note = None
  source 1..21: mol_type = other DNA
gacacgctggtggtgctgcac

SEQ ID NO: 3 - DNA, 21 bp, synthetic construct
  misc_feature 1..21: note = Primer
  source 1..21: mol_type = other DNA
tccactccacaattctgctct

SEQ ID NO: 4 - DNA, 27 bp, synthetic construct
  misc_feature 1..27: note = Primer
  source 1..27: mol_type = other DNA
ttgcttcttatgttaatttggtacaga

SEQ ID NO: 5 - DNA, 19 bp, synthetic construct
  misc_feature 1..19: note = Primer
  source 1..19: mol_type = other DNA
ttgcccatcatcatcacct

SEQ ID NO: 6 - DNA, 21 bp, synthetic construct
  misc_feature 1..21: note = Primer
  source 1..21: mol_type = other DNA
gggttttcttggtgaagttcg

SEQ ID NO: 7 - DNA, 20 bp, synthetic construct
  misc_feature 1..20: note = Primer
  source 1..20: mol_type = other DNA
ctaaggccaaccgtgaaaag

SEQ ID NO: 8 - DNA, 20 bp, synthetic construct
  misc_feature 1..20: note = Primer
  source 1..20: mol_type = other DNA
accagaggcatacagggaca

SEQ ID NO: 9 - DNA, 20 bp, synthetic construct
  misc_feature 1..20: note = Primer
  source 1..20: mol_type = other DNA
acacgtagattccggcaagt

SEQ ID NO: 10 - DNA, 19 bp, synthetic construct
  misc_feature 1..19: note = Primer
  source 1..19: mol_type = other DNA
aggagccctttcccatctc